European Patent Specification EP 3 448 414 B1, published April 17, 2024. Title: NOPE FOR TREATMENT OF PATHOLOGICAL MUSCLE LOSS AND WEAKNESS. Applicant: Five Prime Therapeutics, Inc. GLAXOSMITHKLINE INTELLECTUAL PROPERTY DEVELOPMENT LIMITED Hsu, Amy W. Power, Janine Hinken, Aaron Curtis Russell, Allan James Rocque, Warren James. The sequence listing filed with the application follows.

SEQUENCE LISTING (28 sequences)

SEQ ID NO: 1 - protein, 1250 aa, Artificial Sequence
  Human NOPE precursor (1-1250), with signal peptide.
MARGDAGRGRGLLALTFCLLAARGELLLPQETTVELSCGVGPLQVILGPEQAAVLNCSLGAAAAGPPTRVTWSKDGDTLLEHDHLHLLPNGSLWLSQPLAPNGSDESVPEAVGVIEGNYSCLAHGPLGVLASQTAVVKLATLADFSLHPESQTVEENGTARFECHIEGLPAPIITWEKDQVTLPEEPRLIVLPNGVLQILDVQESDAGPYRCVATNSARQHFSQEALLSVAHRGSLASTRGQDVVIVAAPENTTVVSGQSVVMECVASADPTPFVSWVRQDGKPISTDVIVLGRTNLLIANAQPWHSGVYVCRANKPRTRDFATAAAELRVLAAPAITQAPEALSRTRASTARFVCRASGEPRPALRWLHNGAPLRPNGRVKVQGGGGSLVITQIGLQDAGYYQCVAENSAGMACAAASLAVVVREGLPSAPTRVTATPLSSSAVLVAWERPEMHSEQIIGFSLHYQKARGMDNVEYQFAVNNDTTELQVRDLEPNTDYEFYVVAYSQLGASRTSTPALVHTLDDVPSAAPQLSLSSPNPSDIRVAWLPLPPSLSNGQVVKYKIEYGLGKEDQIFSTEVRGNETQLMLNSLQPNKVYRVRISAGTAAGFGAPSQWMHHRTPSMHNQSHVPFAPAELKVQAKMESLVVSWQPPPHPTQISGYKLYWREVGAEEEANGDRLPGGRGDQAWDVGPVRLKKKVKQYELTQLVPGRLYEVKLVAFNKHEDGYAAVWKGKTEKAPAPDMPIQRGPPLPPAHVHAESNSSTSIWLRWKKPDFTTVKIVNYTVRFSPWGLRNASLVTYYTSSGEDILIGGLKPFTKYEFAVQSHGVDMDGPFGSVVERSTLPDRPSTPPSDLRLSPLTPSTVRLHWCPPTEPNGEIVEYLILYSSNHTQPEHQWTLLTTQGNIFSAEVHGLESDTRYFFKMGARTEVGPGPFSRLQDVITLQEKLSDSLDMHSVTGIIVGVCLGLLCLLACMCAGLRRSPHRESLPGLSSTATPGNPALYSRARLGPPSPPAAHELESLVHPHPQDWSPPPSDVEDRAEVHSLMGGGVSEGRSHSKRKISWAQPSGLSWAGSWAGCELPQAGPRPALTRALLPPAGTGQTLLLQALVYDAIKGNGRKKSPPACRNQVEAEVIVHSDFSASNGNPDLHLQDLEPEDPLPPEAPDLISGVGDPGQGAAWLDRELGGCELAAPGPDRLTCLPEAASASCSYPDLQPGEVLEETPGDSCQLKSPCPLGASPGLPRSPVSSSA

SEQ ID NO: 2 - protein, 1226 aa, Artificial Sequence
  Human mature NOPE (25-1250), without signal peptide.
ELLLPQETTVELSCGVGPLQVILGPEQAAVLNCSLGAAAAGPPTRVTWSKDGDTLLEHDHLHLLPNGSLWLSQPLAPNGSDESVPEAVGVIEGNYSCLAHGPLGVLASQTAVVKLATLADFSLHPESQTVEENGTARFECHIEGLPAPIITWEKDQVTLPEEPRLIVLPNGVLQILDVQESDAGPYRCVATNSARQHFSQEALLSVAHRGSLASTRGQDVVIVAAPENTTVVSGQSVVMECVASADPTPFVSWVRQDGKPISTDVIVLGRTNLLIANAQPWHSGVYVCRANKPRTRDFATAAAELRVLAAPAITQAPEALSRTRASTARFVCRASGEPRPALRWLHNGAPLRPNGRVKVQGGGGSLVITQIGLQDAGYYQCVAENSAGMACAAASLAVVVREGLPSAPTRVTATPLSSSAVLVAWERPEMHSEQIIGFSLHYQKARGMDNVEYQFAVNNDTTELQVRDLEPNTDYEFYVVAYSQLGASRTSTPALVHTLDDVPSAAPQLSLSSPNPSDIRVAWLPLPPSLSNGQVVKYKIEYGLGKEDQIFSTEVRGNETQLMLNSLQPNKVYRVRISAGTAAGFGAPSQWMHHRTPSMHNQSHVPFAPAELKVQAKMESLVVSWQPPPHPTQISGYKLYWREVGAEEEANGDRLPGGRGDQAWDVGPVRLKKKVKQYELTQLVPGRLYEVKLVAFNKHEDGYAAVWKGKTEKAPAPDMPIQRGPPLPPAHVHAESNSSTSIWLRWKKPDFTTVKIVNYTVRFSPWGLRNASLVTYYTSSGEDILIGGLKPFTKYEFAVQSHGVDMDGPFGSVVERSTLPDRPSTPPSDLRLSPLTPSTVRLHWCPPTEPNGEIVEYLILYSSNHTQPEHQWTLLTTQGNIFSAEVHGLESDTRYFFKMGARTEVGPGPFSRLQDVITLQEKLSDSLDMHSVTGIIVGVCLGLLCLLACMCAGLRRSPHRESLPGLSSTATPGNPALYSRARLGPPSPPAAHELESLVHPHPQDWSPPPSDVEDRAEVHSLMGGGVSEGRSHSKRKISWAQPSGLSWAGSWAGCELPQAGPRPALTRALLPPAGTGQTLLLQALVYDAIKGNGRKKSPPACRNQVEAEVIVHSDFSASNGNPDLHLQDLEPEDPLPPEAPDLISGVGDPGQGAAWLDRELGGCELAAPGPDRLTCLPEAASASCSYPDLQPGEVLEETPGDSCQLKSPCPLGASPGLPRSPVSSSA

SEQ ID NO: 3 - protein, 1252 aa, Artificial Sequence
  Mouse NOPE precursor (1-1252), with signal peptide.
MARADTGRGLLVLTFCLLSARGELPLPQETTVKLSCDEGPLQVILGPEQAVVLDCTLGATAAGPPTRVTWSKDGDTVLEHENLHLLPNGSLWLSSPLEQEDSDDEEALRIWKVTEGSYSCLAHSPLGVVASQVAVVKLATLEDFSLHPESQIVEENGTARFECHTKGLPAPIITWEKDQVTVPEESRLITLPNGVLQILDVQDSDAGSYRCVATNSARQRFSQEASLTVALRGSLEATRGQDVVIVAAPENTTVVSGQSVVMECVASADPTPFVSWVRQDGKPISTDVIVLGRTNLLIASAQPRHSGVYVCRANKPRTRDFATAAAELRVLAAPAISQAPEALSRTRASTARFVCRASGEPRPALHWLHDGIPLRPNGRVKVQGGGGSLVITQIGLQDAGYYQCVAENSAGTACAAAPLAVVVREGLPSAPTRVTATPLSSSSVLVAWERPELHSEQIIGFSLHYQKARGVDNVEYQFAVNNDTTELQVRDLEPNTDYEFYVVAYSQLGASRTSSPALVHTLDDVPSAAPQLTLSSPNPSDIRVAWLPLPSSLSNGQVLKYKIEYGLGKEDQVFSTEVPGNETQLTLNSLQPNKVYRVRISAGTGAGYGVPSQWMQHRTPGVHNQSHVPFAPAELKVRAKMESLVVSWQPPPHPTQISGYKLYWREVGTEEEADGDRPPGGRGDQAWDVGPVRLKKKVKQYELTQLVPGRLYEVKLVAFNKHEDGYAAVWKGKTEKAPTPDLPIQRGPPLPPAHVHAESNSSTSIWLRWKKPDFTTVKIVNYTVRFGPWGLRNASLVTYYTSSGEDILIGGLKPFTKYEFAVQSHGVDMDGPFGSVVERSTLPDRPSTPPSDLRLSPLTPSTVRLHWCPPTEPNGEIVEYLILYSNNHTQPEHQWTLLTTEGNIFSAEVHGLESDTRYFFKMGARTEVGPGPFSRLQDVITLQKTFSDSLDVHAVTGIIVGVCLGLLCLLACMCAGLRRSSHREALPGLSSSGTPGNPALYTRARLGPPSVPAAHELESLVHPRPQDWSPPPSDVEDKAEVHSLMGGSVSDCRGHSKRKISWAQAGGPNWAGSWAGCELPQGSGPRPALTRALLPPAGTGQTLLLQALVYDAIKSNGRKKPSPACRNQVEAEVIVHSDFGASKGCPDLHLQDLEPEEPLTAETLPSTSGAVDLSQGADWLGRELGGCQPTTSGPERLTCLPEAASASCSCSDLQPSTAIEEAPGKSCQPKALCPLTVSPSLPRAPVSSAQVP

SEQ ID NO: 4 - protein, 1230 aa, Artificial Sequence
  Mouse mature NOPE (23-1252), without signal peptide.
ELPLPQETTVKLSCDEGPLQVILGPEQAVVLDCTLGATAAGPPTRVTWSKDGDTVLEHENLHLLPNGSLWLSSPLEQEDSDDEEALRIWKVTEGSYSCLAHSPLGVVASQVAVVKLATLEDFSLHPESQIVEENGTARFECHTKGLPAPIITWEKDQVTVPEESRLITLPNGVLQILDVQDSDAGSYRCVATNSARQRFSQEASLTVALRGSLEATRGQDVVIVAAPENTTVVSGQSVVMECVASADPTPFVSWVRQDGKPISTDVIVLGRTNLLIASAQPRHSGVYVCRANKPRTRDFATAAAELRVLAAPAISQAPEALSRTRASTARFVCRASGEPRPALHWLHDGIPLRPNGRVKVQGGGGSLVITQIGLQDAGYYQCVAENSAGTACAAAPLAVVVREGLPSAPTRVTATPLSSSSVLVAWERPELHSEQIIGFSLHYQKARGVDNVEYQFAVNNDTTELQVRDLEPNTDYEFYVVAYSQLGASRTSSPALVHTLDDVPSAAPQLTLSSPNPSDIRVAWLPLPSSLSNGQVLKYKIEYGLGKEDQVFSTEVPGNETQLTLNSLQPNKVYRVRISAGTGAGYGVPSQWMQHRTPGVHNQSHVPFAPAELKVRAKMESLVVSWQPPPHPTQISGYKLYWREVGTEEEADGDRPPGGRGDQAWDVGPVRLKKKVKQYELTQLVPGRLYEVKLVAFNKHEDGYAAVWKGKTEKAPTPDLPIQRGPPLPPAHVHAESNSSTSIWLRWKKPDFTTVKIVNYTVRFGPWGLRNASLVTYYTSSGEDILIGGLKPFTKYEFAVQSHGVDMDGPFGSVVERSTLPDRPSTPPSDLRLSPLTPSTVRLHWCPPTEPNGEIVEYLILYSNNHTQPEHQWTLLTTEGNIFSAEVHGLESDTRYFFKMGARTEVGPGPFSRLQDVITLQKTFSDSLDVHAVTGIIVGVCLGLLCLLACMCAGLRRSSHREALPGLSSSGTPGNPALYTRARLGPPSVPAAHELESLVHPRPQDWSPPPSDVEDKAEVHSLMGGSVSDCRGHSKRKISWAQAGGPNWAGSWAGCELPQGSGPRPALTRALLPPAGTGQTLLLQALVYDAIKSNGRKKPSPACRNQVEAEVIVHSDFGASKGCPDLHLQDLEPEEPLTAETLPSTSGAVDLSQGADWLGRELGGCQPTTSGPERLTCLPEAASASCSCSDLQPSTAIEEAPGKSCQPKALCPLTVSPSLPRAPVSSAQVP

SEQ ID NO: 5 - protein, 957 aa, Artificial Sequence
  Human NOPE extracellular domain (ECD) (1-957), with signal peptide.
MARGDAGRGRGLLALTFCLLAARGELLLPQETTVELSCGVGPLQVILGPEQAAVLNCSLGAAAAGPPTRVTWSKDGDTLLEHDHLHLLPNGSLWLSQPLAPNGSDESVPEAVGVIEGNYSCLAHGPLGVLASQTAVVKLATLADFSLHPESQTVEENGTARFECHIEGLPAPIITWEKDQVTLPEEPRLIVLPNGVLQILDVQESDAGPYRCVATNSARQHFSQEALLSVAHRGSLASTRGQDVVIVAAPENTTVVSGQSVVMECVASADPTPFVSWVRQDGKPISTDVIVLGRTNLLIANAQPWHSGVYVCRANKPRTRDFATAAAELRVLAAPAITQAPEALSRTRASTARFVCRASGEPRPALRWLHNGAPLRPNGRVKVQGGGGSLVITQIGLQDAGYYQCVAENSAGMACAAASLAVVVREGLPSAPTRVTATPLSSSAVLVAWERPEMHSEQIIGFSLHYQKARGMDNVEYQFAVNNDTTELQVRDLEPNTDYEFYVVAYSQLGASRTSTPALVHTLDDVPSAAPQLSLSSPNPSDIRVAWLPLPPSLSNGQVVKYKIEYGLGKEDQIFSTEVRGNETQLMLNSLQPNKVYRVRISAGTAAGFGAPSQWMHHRTPSMHNQSHVPFAPAELKVQAKMESLVVSWQPPPHPTQISGYKLYWREVGAEEEANGDRLPGGRGDQAWDVGPVRLKKKVKQYELTQLVPGRLYEVKLVAFNKHEDGYAAVWKGKTEKAPAPDMPIQRGPPLPPAHVHAESNSSTSIWLRWKKPDFTTVKIVNYTVRFSPWGLRNASLVTYYTSSGEDILIGGLKPFTKYEFAVQSHGVDMDGPFGSVVERSTLPDRPSTPPSDLRLSPLTPSTVRLHWCPPTEPNGEIVEYLILYSSNHTQPEHQWTLLTTQGNIFSAEVHGLESDTRYFFKMGARTEVGPGPFSRLQDVITLQEKLSDSLDMHSVT

SEQ ID NO: 6 - protein, 931 aa, Artificial Sequence
  Human NOPE ECD (25-955), without signal peptide.
ELLLPQETTVELSCGVGPLQVILGPEQAAVLNCSLGAAAAGPPTRVTWSKDGDTLLEHDHLHLLPNGSLWLSQPLAPNGSDESVPEAVGVIEGNYSCLAHGPLGVLASQTAVVKLATLADFSLHPESQTVEENGTARFECHIEGLPAPIITWEKDQVTLPEEPRLIVLPNGVLQILDVQESDAGPYRCVATNSARQHFSQEALLSVAHRGSLASTRGQDVVIVAAPENTTVVSGQSVVMECVASADPTPFVSWVRQDGKPISTDVIVLGRTNLLIANAQPWHSGVYVCRANKPRTRDFATAAAELRVLAAPAITQAPEALSRTRASTARFVCRASGEPRPALRWLHNGAPLRPNGRVKVQGGGGSLVITQIGLQDAGYYQCVAENSAGMACAAASLAVVVREGLPSAPTRVTATPLSSSAVLVAWERPEMHSEQIIGFSLHYQKARGMDNVEYQFAVNNDTTELQVRDLEPNTDYEFYVVAYSQLGASRTSTPALVHTLDDVPSAAPQLSLSSPNPSDIRVAWLPLPPSLSNGQVVKYKIEYGLGKEDQIFSTEVRGNETQLMLNSLQPNKVYRVRISAGTAAGFGAPSQWMHHRTPSMHNQSHVPFAPAELKVQAKMESLVVSWQPPPHPTQISGYKLYWREVGAEEEANGDRLPGGRGDQAWDVGPVRLKKKVKQYELTQLVPGRLYEVKLVAFNKHEDGYAAVWKGKTEKAPAPDMPIQRGPPLPPAHVHAESNSSTSIWLRWKKPDFTTVKIVNYTVRFSPWGLRNASLVTYYTSSGEDILIGGLKPFTKYEFAVQSHGVDMDGPFGSVVERSTLPDRPSTPPSDLRLSPLTPSTVRLHWCPPTEPNGEIVEYLILYSSNHTQPEHQWTLLTTQGNIFSAEVHGLESDTRYFFKMGARTEVGPGPFSRLQDVITLQEKLSDSLDMHS

SEQ ID NO: 7 - protein, 402 aa, Artificial Sequence
  Human NOPE ECD (25-426), without signal peptide.
ELLLPQETTVELSCGVGPLQVILGPEQAAVLNCSLGAAAAGPPTRVTWSKDGDTLLEHDHLHLLPNGSLWLSQPLAPNGSDESVPEAVGVIEGNYSCLAHGPLGVLASQTAVVKLATLADFSLHPESQTVEENGTARFECHIEGLPAPIITWEKDQVTLPEEPRLIVLPNGVLQILDVQESDAGPYRCVATNSARQHFSQEALLSVAHRGSLASTRGQDVVIVAAPENTTVVSGQSVVMECVASADPTPFVSWVRQDGKPISTDVIVLGRTNLLIANAQPWHSGVYVCRANKPRTRDFATAAAELRVLAAPAITQAPEALSRTRASTARFVCRASGEPRPALRWLHNGAPLRPNGRVKVQGGGGSLVITQIGLQDAGYYQCVAENSAGMACAAASLAVVVRE

SEQ ID NO: 8 - protein, 596 aa, Artificial Sequence
  Human NOPE ECD (25-620), without signal peptide.
ELLLPQETTVELSCGVGPLQVILGPEQAAVLNCSLGAAAAGPPTRVTWSKDGDTLLEHDHLHLLPNGSLWLSQPLAPNGSDESVPEAVGVIEGNYSCLAHGPLGVLASQTAVVKLATLADFSLHPESQTVEENGTARFECHIEGLPAPIITWEKDQVTLPEEPRLIVLPNGVLQILDVQESDAGPYRCVATNSARQHFSQEALLSVAHRGSLASTRGQDVVIVAAPENTTVVSGQSVVMECVASADPTPFVSWVRQDGKPISTDVIVLGRTNLLIANAQPWHSGVYVCRANKPRTRDFATAAAELRVLAAPAITQAPEALSRTRASTARFVCRASGEPRPALRWLHNGAPLRPNGRVKVQGGGGSLVITQIGLQDAGYYQCVAENSAGMACAAASLAVVVREGLPSAPTRVTATPLSSSAVLVAWERPEMHSEQIIGFSLHYQKARGMDNVEYQFAVNNDTTELQVRDLEPNTDYEFYVVAYSQLGASRTSTPALVHTLDDVPSAAPQLSLSSPNPSDIRVAWLPLPPSLSNGQVVKYKIEYGLGKEDQIFSTEVRGNETQLMLNSLQPNKVYRVRISAGTAAGFGAPSQWMHHRT

SEQ ID NO: 9 - protein, 529 aa, Artificial Sequence
  Human NOPE ECD (427-955).
GLPSAPTRVTATPLSSSAVLVAWERPEMHSEQIIGFSLHYQKARGMDNVEYQFAVNNDTTELQVRDLEPNTDYEFYVVAYSQLGASRTSTPALVHTLDDVPSAAPQLSLSSPNPSDIRVAWLPLPPSLSNGQVVKYKIEYGLGKEDQIFSTEVRGNETQLMLNSLQPNKVYRVRISAGTAAGFGAPSQWMHHRTPSMHNQSHVPFAPAELKVQAKMESLVVSWQPPPHPTQISGYKLYWREVGAEEEANGDRLPGGRGDQAWDVGPVRLKKKVKQYELTQLVPGRLYEVKLVAFNKHEDGYAAVWKGKTEKAPAPDMPIQRGPPLPPAHVHAESNSSTSIWLRWKKPDFTTVKIVNYTVRFSPWGLRNASLVTYYTSSGEDILIGGLKPFTKYEFAVQSHGVDMDGPFGSVVERSTLPDRPSTPPSDLRLSPLTPSTVRLHWCPPTEPNGEIVEYLILYSSNHTQPEHQWTLLTTQGNIFSAEVHGLESDTRYFFKMGARTEVGPGPFSRLQDVITLQEKLSDSLDMHS

SEQ ID NO: 10 - protein, 333 aa, Artificial Sequence
  Human NOPE ECD (623-955).
MHNQSHVPFAPAELKVQAKMESLVVSWQPPPHPTQISGYKLYWREVGAEEEANGDRLPGGRGDQAWDVGPVRLKKKVKQYELTQLVPGRLYEVKLVAFNKHEDGYAAVWKGKTEKAPAPDMPIQRGPPLPPAHVHAESNSSTSIWLRWKKPDFTTVKIVNYTVRFSPWGLRNASLVTYYTSSGEDILIGGLKPFTKYEFAVQSHGVDMDGPFGSVVERSTLPDRPSTPPSDLRLSPLTPSTVRLHWCPPTEPNGEIVEYLILYSSNHTQPEHQWTLLTTQGNIFSAEVHGLESDTRYFFKMGARTEVGPGPFSRLQDVITLQEKLSDSLDMHS

SEQ ID NO: 11 - protein, 956 aa, Artificial Sequence
  Mouse NOPE extracellular domain (ECD) (1-956), with signal peptide.
MARADTGRGLLVLTFCLLSARGELPLPQETTVKLSCDEGPLQVILGPEQAVVLDCTLGATAAGPPTRVTWSKDGDTVLEHENLHLLPNGSLWLSSPLEQEDSDDEEALRIWKVTEGSYSCLAHSPLGVVASQVAVVKLATLEDFSLHPESQIVEENGTARFECHTKGLPAPIITWEKDQVTVPEESRLITLPNGVLQILDVQDSDAGSYRCVATNSARQRFSQEASLTVALRGSLEATRGQDVVIVAAPENTTVVSGQSVVMECVASADPTPFVSWVRQDGKPISTDVIVLGRTNLLIASAQPRHSGVYVCRANKPRTRDFATAAAELRVLAAPAISQAPEALSRTRASTARFVCRASGEPRPALHWLHDGIPLRPNGRVKVQGGGGSLVITQIGLQDAGYYQCVAENSAGTACAAAPLAVVVREGLPSAPTRVTATPLSSSSVLVAWERPELHSEQIIGFSLHYQKARGVDNVEYQFAVNNDTTELQVRDLEPNTDYEFYVVAYSQLGASRTSSPALVHTLDDVPSAAPQLTLSSPNPSDIRVAWLPLPSSLSNGQVLKYKIEYGLGKEDQVFSTEVPGNETQLTLNSLQPNKVYRVRISAGTGAGYGVPSQWMQHRTPGVHNQSHVPFAPAELKVRAKMESLVVSWQPPPHPTQISGYKLYWREVGTEEEADGDRPPGGRGDQAWDVGPVRLKKKVKQYELTQLVPGRLYEVKLVAFNKHEDGYAAVWKGKTEKAPTPDLPIQRGPPLPPAHVHAESNSSTSIWLRWKKPDFTTVKIVNYTVRFGPWGLRNASLVTYYTSSGEDILIGGLKPFTKYEFAVQSHGVDMDGPFGSVVERSTLPDRPSTPPSDLRLSPLTPSTVRLHWCPPTEPNGEIVEYLILYSNNHTQPEHQWTLLTTEGNIFSAEVHGLESDTRYFFKMGARTEVGPGPFSRLQDVITLQKTFSDSLDVHAVT

SEQ ID NO: 12 - protein, 934 aa, Artificial Sequence
  Mouse NOPE ECD (23-956), without signal peptide.
ELPLPQETTVKLSCDEGPLQVILGPEQAVVLDCTLGATAAGPPTRVTWSKDGDTVLEHENLHLLPNGSLWLSSPLEQEDSDDEEALRIWKVTEGSYSCLAHSPLGVVASQVAVVKLATLEDFSLHPESQIVEENGTARFECHTKGLPAPIITWEKDQVTVPEESRLITLPNGVLQILDVQDSDAGSYRCVATNSARQRFSQEASLTVALRGSLEATRGQDVVIVAAPENTTVVSGQSVVMECVASADPTPFVSWVRQDGKPISTDVIVLGRTNLLIASAQPRHSGVYVCRANKPRTRDFATAAAELRVLAAPAISQAPEALSRTRASTARFVCRASGEPRPALHWLHDGIPLRPNGRVKVQGGGGSLVITQIGLQDAGYYQCVAENSAGTACAAAPLAVVVREGLPSAPTRVTATPLSSSSVLVAWERPELHSEQIIGFSLHYQKARGVDNVEYQFAVNNDTTELQVRDLEPNTDYEFYVVAYSQLGASRTSSPALVHTLDDVPSAAPQLTLSSPNPSDIRVAWLPLPSSLSNGQVLKYKIEYGLGKEDQVFSTEVPGNETQLTLNSLQPNKVYRVRISAGTGAGYGVPSQWMQHRTPGVHNQSHVPFAPAELKVRAKMESLVVSWQPPPHPTQISGYKLYWREVGTEEEADGDRPPGGRGDQAWDVGPVRLKKKVKQYELTQLVPGRLYEVKLVAFNKHEDGYAAVWKGKTEKAPTPDLPIQRGPPLPPAHVHAESNSSTSIWLRWKKPDFTTVKIVNYTVRFGPWGLRNASLVTYYTSSGEDILIGGLKPFTKYEFAVQSHGVDMDGPFGSVVERSTLPDRPSTPPSDLRLSPLTPSTVRLHWCPPTEPNGEIVEYLILYSNNHTQPEHQWTLLTTEGNIFSAEVHGLESDTRYFFKMGARTEVGPGPFSRLQDVITLQKTFSDSLDVHAVT

SEQ ID NO: 13 - protein, 597 aa, Artificial Sequence
  Mouse NOPE ECD (23-619), without signal peptide.
ELPLPQETTVKLSCDEGPLQVILGPEQAVVLDCTLGATAAGPPTRVTWSKDGDTVLEHENLHLLPNGSLWLSSPLEQEDSDDEEALRIWKVTEGSYSCLAHSPLGVVASQVAVVKLATLEDFSLHPESQIVEENGTARFECHTKGLPAPIITWEKDQVTVPEESRLITLPNGVLQILDVQDSDAGSYRCVATNSARQRFSQEASLTVALRGSLEATRGQDVVIVAAPENTTVVSGQSVVMECVASADPTPFVSWVRQDGKPISTDVIVLGRTNLLIASAQPRHSGVYVCRANKPRTRDFATAAAELRVLAAPAISQAPEALSRTRASTARFVCRASGEPRPALHWLHDGIPLRPNGRVKVQGGGGSLVITQIGLQDAGYYQCVAENSAGTACAAAPLAVVVREGLPSAPTRVTATPLSSSSVLVAWERPELHSEQIIGFSLHYQKARGVDNVEYQFAVNNDTTELQVRDLEPNTDYEFYVVAYSQLGASRTSSPALVHTLDDVPSAAPQLTLSSPNPSDIRVAWLPLPSSLSNGQVLKYKIEYGLGKEDQVFSTEVPGNETQLTLNSLQPNKVYRVRISAGTGAGYGVPSQWMQHRT

SEQ ID NO: 14 - protein, 334 aa, Artificial Sequence
  Mouse NOPE ECD (623-956), without signal peptide.
HNQSHVPFAPAELKVRAKMESLVVSWQPPPHPTQISGYKLYWREVGTEEEADGDRPPGGRGDQAWDVGPVRLKKKVKQYELTQLVPGRLYEVKLVAFNKHEDGYAAVWKGKTEKAPTPDLPIQRGPPLPPAHVHAESNSSTSIWLRWKKPDFTTVKIVNYTVRFGPWGLRNASLVTYYTSSGEDILIGGLKPFTKYEFAVQSHGVDMDGPFGSVVERSTLPDRPSTPPSDLRLSPLTPSTVRLHWCPPTEPNGEIVEYLILYSNNHTQPEHQWTLLTTEGNIFSAEVHGLESDTRYFFKMGARTEVGPGPFSRLQDVITLQKTFSDSLDVHAVT

SEQ ID NO: 15 - protein, 1165 aa, Artificial Sequence
  Human NOPE ECD (25-955)-Fc fusion molecule, without signal peptide.
ELLLPQETTVELSCGVGPLQVILGPEQAAVLNCSLGAAAAGPPTRVTWSKDGDTLLEHDHLHLLPNGSLWLSQPLAPNGSDESVPEAVGVIEGNYSCLAHGPLGVLASQTAVVKLATLADFSLHPESQTVEENGTARFECHIEGLPAPIITWEKDQVTLPEEPRLIVLPNGVLQILDVQESDAGPYRCVATNSARQHFSQEALLSVAHRGSLASTRGQDVVIVAAPENTTVVSGQSVVMECVASADPTPFVSWVRQDGKPISTDVIVLGRTNLLIANAQPWHSGVYVCRANKPRTRDFATAAAELRVLAAPAITQAPEALSRTRASTARFVCRASGEPRPALRWLHNGAPLRPNGRVKVQGGGGSLVITQIGLQDAGYYQCVAENSAGMACAAASLAVVVREGLPSAPTRVTATPLSSSAVLVAWERPEMHSEQIIGFSLHYQKARGMDNVEYQFAVNNDTTELQVRDLEPNTDYEFYVVAYSQLGASRTSTPALVHTLDDVPSAAPQLSLSSPNPSDIRVAWLPLPPSLSNGQVVKYKIEYGLGKEDQIFSTEVRGNETQLMLNSLQPNKVYRVRISAGTAAGFGAPSQWMHHRTPSMHNQSHVPFAPAELKVQAKMESLVVSWQPPPHPTQISGYKLYWREVGAEEEANGDRLPGGRGDQAWDVGPVRLKKKVKQYELTQLVPGRLYEVKLVAFNKHEDGYAAVWKGKTEKAPAPDMPIQRGPPLPPAHVHAESNSSTSIWLRWKKPDFTTVKIVNYTVRFSPWGLRNASLVTYYTSSGEDILIGGLKPFTKYEFAVQSHGVDMDGPFGSVVERSTLPDRPSTPPSDLRLSPLTPSTVRLHWCPPTEPNGEIVEYLILYSSNHTQPEHQWTLLTTQGNIFSAEVHGLESDTRYFFKMGARTEVGPGPFSRLQDVITLQEKLSDSLDMHSGSEPKSSDKTHTCPPCPAPELLGGPSVFLFPPKPKDTLMISRTPEVTCVVVDVSHEDPEVKFNWYVDGVEVHNAKTKPREEQYNSTYRVVSVLTVLHQDWLNGKEYKCKVSNKALPAPIEKTISKAKGQPREPQVYTLPPSRDELTKNQVSLTCLVKGFYPSDIAVEWESNGQPENNYKTTPPVLDSDGSFFLYSKLTVDKSRWQQGNVFSCSVMHEALHNHYTQKSLSLSPGK

SEQ ID NO: 16 - protein, 636 aa, Artificial Sequence
  Human NOPE ECD (25-426)-Fc fusion molecule, without signal peptide.
ELLLPQETTVELSCGVGPLQVILGPEQAAVLNCSLGAAAAGPPTRVTWSKDGDTLLEHDHLHLLPNGSLWLSQPLAPNGSDESVPEAVGVIEGNYSCLAHGPLGVLASQTAVVKLATLADFSLHPESQTVEENGTARFECHIEGLPAPIITWEKDQVTLPEEPRLIVLPNGVLQILDVQESDAGPYRCVATNSARQHFSQEALLSVAHRGSLASTRGQDVVIVAAPENTTVVSGQSVVMECVASADPTPFVSWVRQDGKPISTDVIVLGRTNLLIANAQPWHSGVYVCRANKPRTRDFATAAAELRVLAAPAITQAPEALSRTRASTARFVCRASGEPRPALRWLHNGAPLRPNGRVKVQGGGGSLVITQIGLQDAGYYQCVAENSAGMACAAASLAVVVREGSEPKSSDKTHTCPPCPAPELLGGPSVFLFPPKPKDTLMISRTPEVTCVVVDVSHEDPEVKFNWYVDGVEVHNAKTKPREEQYNSTYRVVSVLTVLHQDWLNGKEYKCKVSNKALPAPIEKTISKAKGQPREPQVYTLPPSRDELTKNQVSLTCLVKGFYPSDIAVEWESNGQPENNYKTTPPVLDSDGSFFLYSKLTVDKSRWQQGNVFSCSVMHEALHNHYTQKSLSLSPGK

SEQ ID NO: 17 - protein, 830 aa, Artificial Sequence
  Human NOPE ECD (25-620)-Fc fusion molecule, without signal peptide.
ELLLPQETTVELSCGVGPLQVILGPEQAAVLNCSLGAAAAGPPTRVTWSKDGDTLLEHDHLHLLPNGSLWLSQPLAPNGSDESVPEAVGVIEGNYSCLAHGPLGVLASQTAVVKLATLADFSLHPESQTVEENGTARFECHIEGLPAPIITWEKDQVTLPEEPRLIVLPNGVLQILDVQESDAGPYRCVATNSARQHFSQEALLSVAHRGSLASTRGQDVVIVAAPENTTVVSGQSVVMECVASADPTPFVSWVRQDGKPISTDVIVLGRTNLLIANAQPWHSGVYVCRANKPRTRDFATAAAELRVLAAPAITQAPEALSRTRASTARFVCRASGEPRPALRWLHNGAPLRPNGRVKVQGGGGSLVITQIGLQDAGYYQCVAENSAGMACAAASLAVVVREGLPSAPTRVTATPLSSSAVLVAWERPEMHSEQIIGFSLHYQKARGMDNVEYQFAVNNDTTELQVRDLEPNTDYEFYVVAYSQLGASRTSTPALVHTLDDVPSAAPQLSLSSPNPSDIRVAWLPLPPSLSNGQVVKYKIEYGLGKEDQIFSTEVRGNETQLMLNSLQPNKVYRVRISAGTAAGFGAPSQWMHHRTGSEPKSSDKTHTCPPCPAPELLGGPSVFLFPPKPKDTLMISRTPEVTCVVVDVSHEDPEVKFNWYVDGVEVHNAKTKPREEQYNSTYRVVSVLTVLHQDWLNGKEYKCKVSNKALPAPIEKTISKAKGQPREPQVYTLPPSRDELTKNQVSLTCLVKGFYPSDIAVEWESNGQPENNYKTTPPVLDSDGSFFLYSKLTVDKSRWQQGNVFSCSVMHEALHNHYTQKSLSLSPGK

SEQ ID NO: 18 - protein, 763 aa, Artificial Sequence
  Human NOPE ECD (427-955)-Fc fusion molecule, without signal peptide.
GLPSAPTRVTATPLSSSAVLVAWERPEMHSEQIIGFSLHYQKARGMDNVEYQFAVNNDTTELQVRDLEPNTDYEFYVVAYSQLGASRTSTPALVHTLDDVPSAAPQLSLSSPNPSDIRVAWLPLPPSLSNGQVVKYKIEYGLGKEDQIFSTEVRGNETQLMLNSLQPNKVYRVRISAGTAAGFGAPSQWMHHRTPSMHNQSHVPFAPAELKVQAKMESLVVSWQPPPHPTQISGYKLYWREVGAEEEANGDRLPGGRGDQAWDVGPVRLKKKVKQYELTQLVPGRLYEVKLVAFNKHEDGYAAVWKGKTEKAPAPDMPIQRGPPLPPAHVHAESNSSTSIWLRWKKPDFTTVKIVNYTVRFSPWGLRNASLVTYYTSSGEDILIGGLKPFTKYEFAVQSHGVDMDGPFGSVVERSTLPDRPSTPPSDLRLSPLTPSTVRLHWCPPTEPNGEIVEYLILYSSNHTQPEHQWTLLTTQGNIFSAEVHGLESDTRYFFKMGARTEVGPGPFSRLQDVITLQEKLSDSLDMHSGSEPKSSDKTHTCPPCPAPELLGGPSVFLFPPKPKDTLMISRTPEVTCVVVDVSHEDPEVKFNWYVDGVEVHNAKTKPREEQYNSTYRVVSVLTVLHQDWLNGKEYKCKVSNKALPAPIEKTISKAKGQPREPQVYTLPPSRDELTKNQVSLTCLVKGFYPSDIAVEWESNGQPENNYKTTPPVLDSDGSFFLYSKLTVDKSRWQQGNVFSCSVMHEALHNHYTQKSLSLSPGK

SEQ ID NO: 19 - protein, 567 aa, Artificial Sequence
  Human NOPE ECD (623-955)-Fc fusion molecule, without signal peptide.
MHNQSHVPFAPAELKVQAKMESLVVSWQPPPHPTQISGYKLYWREVGAEEEANGDRLPGGRGDQAWDVGPVRLKKKVKQYELTQLVPGRLYEVKLVAFNKHEDGYAAVWKGKTEKAPAPDMPIQRGPPLPPAHVHAESNSSTSIWLRWKKPDFTTVKIVNYTVRFSPWGLRNASLVTYYTSSGEDILIGGLKPFTKYEFAVQSHGVDMDGPFGSVVERSTLPDRPSTPPSDLRLSPLTPSTVRLHWCPPTEPNGEIVEYLILYSSNHTQPEHQWTLLTTQGNIFSAEVHGLESDTRYFFKMGARTEVGPGPFSRLQDVITLQEKLSDSLDMHSGSEPKSSDKTHTCPPCPAPELLGGPSVFLFPPKPKDTLMISRTPEVTCVVVDVSHEDPEVKFNWYVDGVEVHNAKTKPREEQYNSTYRVVSVLTVLHQDWLNGKEYKCKVSNKALPAPIEKTISKAKGQPREPQVYTLPPSRDELTKNQVSLTCLVKGFYPSDIAVEWESNGQPENNYKTTPPVLDSDGSFFLYSKLTVDKSRWQQGNVFSCSVMHEALHNHYTQKSLSLSPGK

SEQ ID NO: 20 - protein, 109 aa, Artificial Sequence
  Human myostatin.
DFGLDCDEHSTESRCCRYPLTVDFEAFGWDWIIAPKRYKANYCSGECEFVFLQKYPHTHLVHQANPRGSAGPCCTPTKMSPINMLYFNGKEQIIYGKIPAMVVDRCGCS

SEQ ID NO: 21 - protein, 375 aa, Artificial Sequence
  Human pro-myostatin (with signal sequence).
MQKLQLCVYIYLFMLIVAGPVDLNENSEQKENVEKEGLCNACTWRQNTKSSRIEAIKIQILSKLRLETAPNISKDVIRQLLPKAPPLRELIDQYDVQRDDSSDGSLEDDDYHATTETIITMPTESDFLMQVDGKPKCCFFKFSSKIQYNKVVKAQLWIYLRPVETPTTVFVQILRLIKPMKDGTRYTGIRSLKLDMNPGTGIWQSIDVKTVLQNWLKQPESNLGIEIKALDENGHDLAVTFPGPGEDGLNPFLEVKVTDTPKRSRRDFGLDCDEHSTESRCCRYPLTVDFEAFGWDWIIAPKRYKANYCSGECEFVFLQKYPHTHLVHQANPRGSAGPCCTPTKMSPINMLYFNGKEQIIYGKIPAMVVDRCGCS

SEQ ID NO: 22 - protein, 352 aa, Artificial Sequence [sequence omitted]

SEQ ID NO: 23 - protein, 109 aa, Artificial Sequence; identical to SEQ ID NO: 20
  Mouse myostatin.

SEQ ID NO: 24 - protein, 376 aa, Artificial Sequence
  Mouse pro-myostatin (with signal sequence).
MMQKLQMYVYIYLFMLIAAGPVDLNEGSEREENVEKEGLCNACAWRQNTRYSRIEAIKIQILSKLRLETAPNISKDAIRQLLPRAPPLRELIDQYDVQRDDSSDGSLEDDDYHATTETIITMPTESDFLMQADGKPKCCFFKFSSKIQYNKVVKAQLWIYLRPVKTPTTVFVQILRLIKPMKDGTRYTGIRSLKLDMSPGTGIWQSIDVKTVLQNWLKQPESNLGIEIKALDENGHDLAVTFPGPGEDGLNPFLEVKVTDTPKRSRRDFGLDCDEHSTESRCCRYPLTVDFEAFGWDWIIAPKRYKANYCSGECEFVFLQKYPHTHLVHQANPRGSAGPCCTPTKMSPINMLYFNGKEQIIYGKIPAMVVDRCGCS

SEQ ID NO: 25 - protein, 351 aa, Artificial Sequence
  Mouse pro-myostatin (without signal sequence).
EGSEREENVEKEGLCNACAWRQNTRYSRIEAIKIQILSKLRLETAPNISKDAIRQLLPRAPPLRELIDQYDVQRDDSSDGSLEDDDYHATTETIITMPTESDFLMQADGKPKCCFFKFSSKIQYNKVVKAQLWIYLRPVKTPTTVFVQILRLIKPMKDGTRYTGIRSLKLDMSPGTGIWQSIDVKTVLQNWLKQPESNLGIEIKALDENGHDLAVTFPGPGEDGLNPFLEVKVTDTPKRSRRDFGLDCDEHSTESRCCRYPLTVDFEAFGWDWIIAPKRYKANYCSGECEFVFLQKYPHTHLVHQANPRGSAGPCCTPTKMSPINMLYFNGKEQIIYGKIPAMVVDRCGCS

SEQ ID NO: 26 - protein, 232 aa, Artificial Sequence
  Fc C237S.
EPKSSDKTHTCPPCPAPELLGGPSVFLFPPKPKDTLMISRTPEVTCVVVDVSHEDPEVKFNWYVDGVEVHNAKTKPREEQYNSTYRVVSVLTVLHQDWLNGKEYKCKVSNKALPAPIEKTISKAKGQPREPQVYTLPPSRDELTKNQVSLTCLVKGFYPSDIAVEWESNGQPENNYKTTPPVLDSDGSFFLYSKLTVDKSRWQQGNVFSCSVMHEALHNHYTQKSLSLSPGK

SEQ ID NO: 27 - protein, 228 aa, Artificial Sequence
  Exemplary Fc #1.
ERKCCVECPPCPAPPVAGPSVFLFPPKPKDTLMISRTPEVTCVVVDVSHEDPEVQFNWYVDGVEVHNAKTKPREEQFNSTFRVVSVLTVVHQDWLNGKEYKCKVSNKGLPAPIEKTISKTKGQPREPQVYTLPPSREEMTKNQVSLTCLVKGFYPSDIAVEWESNGQPENNYKTTPPMLDSDGSFFLYSKLTVDKSRWQQGNVFSCSVMHEALHNHYTQKSLSLSPGK

SEQ ID NO: 28 - protein, 229 aa, Artificial Sequence
  Exemplary Fc #2.
ESKYGPPCPSCPAPEFLGGPSVFLFPPKPKDTLMISRTPEVTCVVVDVSQEDPEVQFNWYVDGVEVHNAKTKPREEQFNSTYRVVSVLTVLHQDWLNGKEYKCKVSNKGLPSSIEKTISKAKGQPREPQVYTLPPSQEEMTKNQVSLTCLVKGFYPSDIAVEWESNGQPENNYKTTPPVLDSDGSFFLYSRLTVDKSRWQEGNVFSCSVMHEALHNHYTQKSLSLSLGK